European Patent Specification EP 3 200 820 B1, published July 5, 2023. Title: Broad-spectrum vaccine against avian Reovirus. Applicant: Intervet International BV. The sequence listing filed with the application follows.

SEQUENCE LISTING (20 sequences)

SEQ ID NO: 1 - protein, 315 aa, Avian orthoreovirus
  misc_feature (168)..(168): Xaa can be any naturally occurring amino acid
MAGLNPLQRREVVSLILSLTSNVTTNPGDLKSIHERLTSLEASTESLHQSVSGMSATLSGLSADLQDTTRTLDDVTVTLNGLSATIAALQNSLTTLSATVDELANTSSAHSGMLSSLQTAVNGNSSDIANLRSDVSANGLNITDLQNRIKSLESDTSHCLSFSPPLSXADGVVSLDMDPYFCSQRVSLTSYSAEAQLMQFQWVAKGTSGSSDTIDMIVNAHCHGRRTDYIMSSTGSLTVTSNAVSLTFDLSYITNMPSDLSRLIPSAGFQVASFPVDVSFTRESSTHTYQSYGAYSSARVFTITFPTGGNGTSNI

SEQ ID NO: 2 - protein, 309 aa, Avian orthoreovirus
  misc_feature (137)..(137): Xaa can be any naturally occurring amino acid
MAGLTPSQRREVVGLILSLTSSATTSCGDLTAINERLLKLDSSVESLTISVGDLSRRFSELEVDLQNVDSSLRQLTSSLNTLSEEVRQLRSAVSDNTVSISGLSATVADHQQVLTDLQTSVNANVTDITNLKGSVTXLSLTVADLEKRLKVVESGSSSTLEFTSPLSLTNGVVSLNMDPYFCSDNHALTSYSSDAQLMQFQWLARGDDGSSDSVEMLVNAHCHGRRTDYMMSTTENLTVTGNSTSLVFSLEYITKPPSDMSRLVPRAGFQAASFPVDVSFTRDTATHAYQVYGAFTSPRVFKITFLTGG

SEQ ID NO: 3 - protein, 313 aa, Avian orthoreovirus
MAGLTPSQRREVVGLILSLTSNASINPGDLAPIYSRLTALEVARDELNKSLTELSSAMSAFSIRFDDALMKLNSVTADLTVIKSDISTLNSSVSAVTSSTAGLSQSVSSHESQLATLSSSLTTLSSQMAALQRDVSTSELKLTDLQHRVTALESSGGASLQFLPPLKTDGTSVSLELDPYFCSERHNLTSYSAAAQLLQFQWLIRSENGASDSFDMNVVAHCHGRRTDYLMSTPSSLTVTSNSVSLVFDLSFITTPQVDLARLVPCHGFQQATFPVDVSYTRGDTTHSYQVYGSFDTPRIFKITFSTGGTGTA

SEQ ID NO: 4 - protein, 315 aa, Avian orthoreovirus
MEGLTQSQRREVVGLILSLTSSVTTSTGDLAQIRSRLSALESSNALLSETVNGALSQLVALSSRLDNLAATVADGQLELRSLTTDVKNIRSLLDDISTTVASLSASVHKHDLSISDLARQFGLLTTDTANLKTDVATQSLQITSLEQRVTALESGTGSLPSFSAPLKLDDGTVSLDLDPYFCSVDHNLTSYSASAQLMQFQWLVRGEGGSSDSIDMNVTAHCHGRRTDYMMSTTQSLTVTGTSVSLVFNLDTLITSPSDYSRLIPCHGFQQATFPVDLSFKRDEVTHSYQVYGSYSTPRVFKVTFSPGAPVPAVI

SEQ ID NO: 5 - protein, 316 aa, Avian orthoreovirus
MAGLNPSQRREVVSLILSLTSSTTTSPGDLIQIRERLSALESANALLNESVNTALSKLGDFSVALDNMAVNVAETKVELASLASDVQSLRTSLDSTASEVASLSLLVHGHGSSISDLQQKGYALSGEVDNLKSSVSSQGLTISGLESQVQALESGSGTDLLFADPLKLEAGTVSLDLDPYFCSVSRNLTSYSASAQLMQFQWSVKGEDGAANSIDMDVNAHCHGPRTDYLMSTKQSLTVTTSPATLVFELDRIVTLPPDLSRLIPCHAFQQATFPVDISFQREGVSHTYQVYGTYTSSRVFRITFSPGSPGPTVIQ

SEQ ID NO: 6 - protein, 309 aa, Avian orthoreovirus
MAGLNPSQRREVVSLILSLTSNVTISHGDLTPIYERLTNLEASTELLHRSISDISTTVSNISANLQDMTHTLDDVTANLDGLRTTVTALQDSVSILSTNVTDLTNTSSAHAATLSSLQTTVDENSTAISNLKSDVSSNGLAITDLQDRVKSLESTASHGLSFSPPLSVADGVVSLDMDPYFCSQRVSLTSYSAEAQLMQFRWMARGTNGSSDTIDMTVNAHCHGRRTDYMMSSTGNLTVTSNVVLLTFDLSYITPIPSDLARLVSQCGIPSCVVPCGRIIHPRFCDSCVPSVWGVLELTCLHNYFPNRR

SEQ ID NO: 7 - protein, 314 aa, Avian orthoreovirus
MAGLNPLQRREVVSLILSLTSNVNTNPGDLTSVYERLTGLEASTESLHQSVSSMAATVSDISADLQGTTRALDDVTVTLKSLSTSITTLQNSVTTLSATVAELTDTSSAHSGTLSSLQTTVSGNSNAIASLKSDVSANSLSITDLQNRVKSLESGTSHGLSFSPPLNIANGVVSLDMDPYFCSQRVSLTSYSAEAQLMQFQWVARGTTGSSDTIDMTVNAHCHGRRTDYMMSSTGGLTVASNAVSLTFDLDYITNMPPDLSRLIPSAGFQAASFPVDISFTRDSSTHTYQVYGVYSSSRVFTITFPTGGNGTTN

SEQ ID NO: 8 - protein, 314 aa, Avian orthoreovirus
  misc_feature (61)..(61): Xaa can be any naturally occurring amino acid
  misc_feature (66)..(66): Xaa can be any naturally occurring amino acid
  misc_feature (130)..(130): Xaa can be any naturally occurring amino acid
  misc_feature (286)..(286): Xaa can be any naturally occurring amino acid
  misc_feature (308)..(308): Xaa can be any naturally occurring amino acid
  misc_feature (310)..(310): Xaa can be any naturally occurring amino acid
MAGLNPLQRREVVGLILSLTSNVTTNPGDLKSIHERLTSLEASTESLHQSVSSMSATLSDXSADLXDTTRALDDVTVTMNSLSATIAALQNSLTTLSATVDELTDTSSAHSGMLSSLQTTVNGNSSAISXLRSDVSANGLNITDLQNRVKSLESDTSHGLSFSPPLSVADGVVSLSMDPYFCSQRVSLTSYSAEAQLMQFQWVAKGTSGSSDTIDMTVNAHCHGRRTDYMMSSTGGLTVTSNAVSLTFDLNYITNMPSDLSRLIPSAGFQVASFPVDVSFTRESSXHTYQVYGAYSSARVFTITFPTXVXHIKH

SEQ ID NO: 9 - protein, 314 aa, Avian orthoreovirus
MAGLTPLQRREVVGLILSLTSSGNTNCGDLTPIYDRLSSLESAVASLNGSVNGLLQKVPDLETDLQNVVSSLDQTNSTLAELSKELRQLSSSVDNVVTSISDISTTVSGHQDAITAIQISVHANTTAITNLKSSASTASLKITDLERRVEAIESGSDSNLRFVSPLSLSQGVVSLVMDPYFCSDNQALTSYSTDAQLMQFQWLARGDDGSSSSVDMLVNAHCHGRRTDYMMSTTESFTVTGNSVSLVFNLDYITKPPTEMSRLIPRAGFRAASFPVDVSFTRDTTTHAYQVYGAFSSARVFKITFLTGALGRQF

SEQ ID NO: 10 - protein, 312 aa, Avian orthoreovirus
MAGLTPLQRREVVGLILSLTSSGNTNCGDLTPIYDRLSSLESAVASLNGSVNGLLQKVPDLETDLQNVVSSLDQTNSTLAELSKELRQLSSSVDNVVTSISGISTTVSGHQDAITAIQISVHANTTAITNLKSSASTASLKITDLERRLEAVESGSDSNLRFVSPLSLSQGVVSLVMDPYFCSDNQALTSYSTDAQLMQFQWLARGDDGSSSSVDMLVNAHCHGRRTDYMMSTTESFTVTGNSVSLVFNLDYITKPPTDMSRLIPRAGFRAASFPVDVSFTRDTTTHAYQVYGAFSSARVFKITFLTGGTGT

SEQ ID NO: 11 - protein, 315 aa, Avian orthoreovirus
MAGLTPLQRREVVGLILSLTSNATTNCGDLTAIYNRLLKLDSSVESLTTSVGELSKQFLALESGFQNVESSIGQLNTSFDTLSEEARQLQSSVTDITNSISSLSATVSEHQNSLAALQTSVQTNITDIANLKSSVTTLSLTATDLERRLKVIESGSSSSLTFSSPLSLSNGVVSLNMDPYFCSDNYALTSYSSDAQLMQFQWLARGGDGSSGSVEMLVNAHCHGRRTDYMMSTTENLTVTGNSTSLVFSLEYITKPPSDMSRLIPRAGFQAASFPVDVSFTRDTATHAYQVYGVFTTPRIFKITFLTGGTGAAKF

SEQ ID NO: 12 - protein, 306 aa, Avian orthoreovirus
  misc_feature (303)..(303): Xaa can be any naturally occurring amino acid
MEGLTPLQRREVVGLILSLTSSVSISPGDLIPLYERLSAVEETCATVNDSLGRLTSLVSEISARIDDLARTLQDTAAGLDGVQGHVTTLQSSFDDLFSRVATLSSSVSNQESHLTTISASVSTLSTHVSNLQHDVSSTALTVTSLEHRVEALESGAGSDLTFMAPLKVDGKSVSLDLDPYFCSERTNLTSYSANAQLLQFQWLVRSEGGSSDSIDMNVVAHCHGRRTDYLMSTHDSLTVVGNSVTLIFNLDFITTQGVDYARLVPCHGFQQATFPVDISFTKGTATQSYQVYGAFDGPRIFKXTFS

SEQ ID NO: 13 - protein, 313 aa, Avian orthoreovirus
MAGLTPSQRREVVGLILSLTSNTSINPGDLAPIYSRLTALEVARDELNESLSELSSAVSALSTRFDDASMKLNSITADLTVIKSDISVLNSSVSGVTSSMAALSQSVSNHESQLATLSSSLATLSSQVAALQRDVSASELKLTDLQHRVTALESSGGTSLRFLPPFKTDGASVSLELDPYFCSERHNLTSYSAAAQLLQFQWLVKGESGVSDSFDMNVVAHCHGRRTDYLMFTPSSLTVTSNSVSLVFDLSFIITPQIDLARLVPCYGFQQATFPVDVSYTRGEDTHSYQVYGSFDTPRIFKITFSTGGTGTA

SEQ ID NO: 14 - protein, 276 aa, Avian orthoreovirus
MDGLTQSQRREVVGLILSLTSNVTINPGDLLQLRNRVSALESATASLNETVKATLDQLVDLSQKLSNAAAAVVEIRRDLSSLTGDVQVVQSSLESLTDDMSDLSNQVNVSASSITSLTSRVDGLTVDVTNLKSDVSKQGLKLNGLEQRVANLENDTGSAYTFAAPLKLDNGTVSLDLDPYFCSVDRNLTSYSASALLMNFQWLVRGEGGSSDSIDMNVTAHSHGQRTDYMMSTTQSLTVTGNSVSLVFDLDALMSPPTDYSRLIPCHGFQQATFPS

SEQ ID NO: 15 - protein, 315 aa, Avian orthoreovirus
MDGLTQSQRREVVGLILSLTSNVTINPGDLLQLRNRVSVLESATASLNETVRATLDQLVDLSQKLSNAAAAVVEIRRDLSSLTGDVQVVQSSLESLTDDTSDLSNQMNVSASSITSLTSRVDGLTVDVTNLKSDVSKQGLTLSGLEQRVVNLENDTGSAHTFAAPLKLDNGTVSLDLDPYFCSVDHNLTSYSASALLMNFQWLVRGEGGSSDSIDMNVTAHSHGQRTDYMMSTTQSLTVTGNSVSLVFDLDALISPPTDYSRLIPCHGFQQATFPVDLSFKRDDAAYSYQVYGSFTSPRVFKITFSPGNSVPAVI

SEQ ID NO: 16 - protein, 318 aa, Avian orthoreovirus
MDGLTQSQRREVVRLILSLTSNVTINPGDLTQLRERVSALESANASLNETIRAVLDQLVDLSQQLGHAVAAVVEMRRDLNSLTGDVQTVQSSLGPLTDSVSDLSSRVTESSSSITNLLGRVDRLTTDVTNLKSDVSDQGLKVSSLEQRVTNLETGTGSVYTFAAPLKLDGGTVSLDLDPYFCSVDHNLTSYSASAQLMNFQWLVRGEGGSSDSIDMNVTAHSHGQRTDYMMSTTQSLTVTGNPVSLVFDLNALTSPPSDYSRLIPCHGFQQATFPVDLSFKRDDVTYSYQVYGSYTSPRVFKITFSPGNPVPAIIRFI

SEQ ID NO: 17 - protein, 314 aa, Avian orthoreovirus
MDGLTQQQRREVVGLILSLTSSVTINPGDLTQIRERLSALESSNASLSESVGAVSSKLADLSVVLDNMAVSVAETRLELSSVISDVQSLRSSLDSSISELASISSLVHDHSSSISGLQRDNGALSNEVGNLKSSVSSQGLTVSSLERRVQSLEGSSSMNLSFADPLKLENGTVSLELDPYFCSVSRNLTSYSADAQLMQFQWSVKGEDGAGNSIDMDVNAHCHGSRTDYLMSTKQSLTVTTSPATLVFELDRIVSLPSDLSRLVPCYGFQQATFPVDISFQRDGVSHTYQVYGTYTSSRVFKITFSPGTPGPTG

SEQ ID NO: 18 - protein, 315 aa, Avian orthoreovirus
  misc_feature (314)..(314): Xaa can be any naturally occurring amino acid
MDGLTQQQRREVVGLILSLTSSVTINPGDLIQIRERLSALESANVSLNESVDMVLSKLSDLSVALDNMAVSVAEMRVGLSSLTSDVQGLRASLDSSASELTSLSLSVQGHSSLISDLQREGRALSVEVDNLKSSVSSHGLTISSLEQRVQALEVGSSASLSFTDPLKLEAGTVSLDLDPYFCSVNRNLTSYSASAQLMSFQWSVKGEDGASNSIDMDVNAHCHGSRTDYLMSTKQSLTVLTSPATLVFELDRIINIPSDLSRLIPCHGFRQATFPVDISFQRDGASHTYQVYGTFTSSRAFKITFSPGSSGPAXF

SEQ ID NO: 19 - DNA, 20 bp, Artificial Sequence
  PCR primer
agtatttgtgagtacgattg

SEQ ID NO: 20 - DNA, 17 bp, Artificial Sequence
  PCR primer
ggcgccacaccttaggt